European Patent Application EP 4 748 860 A1, published May 27, 2026. Title: 一种抗HER2纳米抗体及其制备方法和应用. Applicant: 康立泰生物医药（青岛）有限公司. The sequence listing filed with the application follows.

SEQUENCE LISTING (102 sequences)

SEQ ID NO: 1 - protein, 630 aa, synthetic construct
  source 1..630: note = HER2-His recombinant protein
TQVCTGTDMKLRLPASPETHLDMLRHLYQGCQVVQGNLELTYLPTNASLSFLQDIQEVQGYVLIAHNQVRQVPLQRLRIVRGTQLFEDNYALAVLDNGDPLNNTTPVTGASPGGLRELQLRSLTEILKGGVLIQRNPQLCYQDTILWKDIFHKNNQLALTLIDTNRSRACHPCSPMCKGSRCWGESSEDCQSLTRTVCAGGCARCKGPLPTDCCHEQCAAGCTGPKHSDCLACLHFNHSGICELHCPALVTYNTDTFESMPNPEGRYTFGASCVTACPYNYLSTDVGSCTLVCPLHNQEVTAEDGTQRCEKCSKPCARVCYGLGMEHLREVRAVTSANIQEFAGCKKIFGSLAFLPESFDGDPASNTAPLQPEQLQVFETLEEITGYLYISAWPDSLPDLSVFQNLQVIRGRILHNGAYSLTLQGLGISWLGLRSLRELGSGLALIHHNTHLCFVHTVPWDQLFRNPHQALLHTANRPEDECVGEGLACHQLCARGHCWGPGPTQCVNCSQFLRGQECVEECRVLQGLPREYVNARHCLPCHPECQPQNGSVTCFGPEADQCVACAHYKDPPFCVARCPSGVKPDLSYMPIWKFPDEEGACQPCPINCTHSCVDLDDKGCPAEQRASPLT

SEQ ID NO: 2 - DNA, 23 bp, synthetic construct
  source 1..23: mol_type = other DNA; note = Forward primer F1
gtcctggctgctcttctacaagg

SEQ ID NO: 3 - DNA, 23 bp, synthetic construct
  source 1..23: mol_type = other DNA; note = Reverse primer R1
ggtacgtgctgttgaactgttcc

SEQ ID NO: 4 - DNA, 35 bp, synthetic construct
  source 1..35: mol_type = other DNA; note = Forward primer F2
atggcccaggtgcagctgcaggagtctggrggagg

SEQ ID NO: 5 - DNA, 27 bp, synthetic construct
  source 1..27: mol_type = other DNA; note = Reverse primer R2
gtggtgtgaggagacggtgacctgggt

SEQ ID NO: 6 - protein, 127 aa, synthetic construct
  source 1..127: note = HER2-1 VHH sequence
QVQLQESGGGLVQAEGSLRLSCAASGRTFSTYDIGWFRQAPGKEREFVARITRYGTGPLYAGSVKGRFTISRDNAKNTVYLQMNGLKPEDTAVYYCAVQSGIGRVYDYRASVSYTYWGQGTQVTVSS

SEQ ID NO: 7 - protein, 119 aa, synthetic construct
  source 1..119: note = HER2-2 VHH sequence
QVQLQESGGGLVQAGDSLRLSCAASGLTFSTVGMGWFRQLLGKEREPVAAISWTGNVIGYGDSVKGRFTISRDSAKNTVYLQMNSLKPEDTAVYYCAARRRGTSSYDYWGQGTQVTVSS

SEQ ID NO: 8 - protein, 119 aa, synthetic construct
  source 1..119: note = HER2-3 VHH sequence
QVQLQESGGGLVQAGDSLRLSCAASGLTFSTVGMGWFRQVLGMEREPVAGISWTGNVIGYAESVTGRFTISRDSAKNTVYLQMNSLKPEDTAVYYCAARRRGMSSYDYWGQGTQVTVSS

SEQ ID NO: 9 - protein, 127 aa, synthetic construct
  source 1..127: note = HER2-4 VHH sequence
QVQLQESGGGLVPAEGSLRLSCAASGRTFIPYDIGWFRQAPGKEREFVAHINRLGIGALYAGSVEGRVTISRDNVKNTVYLQMNGLKPEDTAVYYCAAQSGIGAIYDYRASVSYTYWGQGTQVTVSS

SEQ ID NO: 10 - protein, 121 aa, synthetic construct
  source 1..121: note = HER2-5 VHH sequence
QVQLQESGGGLVQAGDSLRLSCAASERTFARYVMGWFRQAPGKDREFVAHIYSSGSTAYEGSVKGRFTISRDNAKNTVYLQMNSLKPEDTAVYYCAARDRDSTWNQGTSHWGQGTQVTVSS

SEQ ID NO: 11 - protein, 127 aa, synthetic construct
  source 1..127: note = HER2-8 VHH sequence
QVQLQESGGGLVQAGGSLRLSCAASGRTFSGAGVGWFRQDPEKEREFVAAIAWSGGSTRYADSVKGRFTISRDNTENTVFLQMNNLRPEDTAVYYCAATRRFYSGLTYTQRDVYDNWGQGTQVTVSS

SEQ ID NO: 12 - protein, 113 aa, synthetic construct
  source 1..113: note = HER2-10 VHH sequence
QVQLQESGGGLVQPGGSLRLSCTAARNIFGRNVMGWFRQAPGKQREFVAHITGGSAVIYATSVKGRFTISRDNAKNTVYLQMNNLTLDDTAVYFCRAVNDDLWGQGTQVTVSS

SEQ ID NO: 13 - protein, 128 aa, synthetic construct
  source 1..128: note = HER2-11 VHH sequence
QVQLQESGGGLVQAGGSLRLSCAASGHTVSRNMMGWFRQAPGKEREFVSAIAWNGEDTYYAESVEGRFTISKDNVKNTIYLQMNSLKPEDTAVYYCAASLFRLWNSATAGNNRVYHYWGQGTQVTVSS

SEQ ID NO: 14 - protein, 121 aa, synthetic construct
  source 1..121: note = HER2-16 VHH sequence
QVQLQESGGGLVQPGGSLRLSCAPSGSIFAFNAMGWYRQAPGKQRELVATITKEGNTNYVDSVKGRFTISRDNYKNTVDLHMTSLKPDDTAVYYCNARDTRKWVSGGYDYWGQGTQVTVSS

SEQ ID NO: 15 - protein, 123 aa, synthetic construct
  source 1..123: note = HER2-32 VHH sequence
QVQLQESGGGLVQAGGSLRLTCAASGGTISTDVMGWFRQDPGKEREFVAAIQWSRDYTYYSDSVKGRFTGSRDNAKNTVYLQMNSLKPEDAAVYYCARHWSGDIYASNSYNSWGQGTQVTVSS

SEQ ID NO: 16 - protein, 112 aa, synthetic construct
  source 1..112: note = HER2-34 VHH sequence
QVQLQESGGGLVQPGGSLNLSCAASRSIFNALMGWYRQAPGNQREFVAHITRGGSTMYADSVKGRFTISRDNAKNTVYLQMNGLKPDDSAVYYCRDWGHDSWGQGTQVTVSS

SEQ ID NO: 17 - protein, 128 aa, synthetic construct
  source 1..128: note = HER2-37 VHH sequence
QVQLQESGGGLVQAGGSLRLSCAASGRTFSSYDVAWFRQAPEKEREFVAGIRWRGSIAYYVDSVKGRFTISRDNAKNTVYLQMNGLKPEDTAVYYCAATVRTYYGENYDRDASAYGYWGQGTQVTVSS

SEQ ID NO: 18 - protein, 118 aa, synthetic construct
  source 1..118: note = HER2-38 VHH sequence
QLQESGGGLVQAGDSLRLSCAASERTFARYVMGWFRQAPGKDREFVAHIYSSGSTAYEGSVKGRFTISRDNAKNTVYLQMNNLKPEDTAVYYCAARPRDTVWTSSASWGQGTQVTVSS

SEQ ID NO: 19 - protein, 119 aa, synthetic construct
  source 1..119: note = HER2-40 VHH sequence
RVQLQESGGGLVQAGGSMRLSCAASGLTFSTVGMGWFRQLLGKEREPVAAISWTGNVIGYGDSVKGRFTISRDSAKNTVYLQMNSLKPEDTAVYYCAARRRGTSSYDYWGQGTQVTVSS

SEQ ID NO: 20 - protein, 121 aa, synthetic construct
  source 1..121: note = HER2-41 VHH sequence
QVQLQESGGGLVQAGGSLRLSCAASGRIESSYVVGWFRQPPGKEREFVTSIPWSGGATAYAGSVKGRFTISRDNAKNTLYLQMNNLKPEDTAVYYCAARTRDSVWTSSTSWGQGTQVTVSS

SEQ ID NO: 21 - DNA, 39 bp, synthetic construct
  source 1..39: mol_type = other DNA; note = Primer HF
ccttaagggcgtgcagtgccaggtgcagctgcaggagtc

SEQ ID NO: 22 - DNA, 37 bp, synthetic construct
  source 1..37: mol_type = other DNA; note = Primer HR
gatttgggctcgctagctgaggagacggtgacctggg

SEQ ID NO: 23 - protein, 214 aa, synthetic construct
  source 1..214: note = Trastuzumab light chain
DIQMTQSPSSLSASVGDRVTITCRASQDVNTAVAWYQQKPGKAPKLLIYSASFLYSGVPSRFSGSRSGTDFTLTISSLQPEDFATYYCQQHYTTPPTFGQGTKVEIKRTVAAPSVFIFPPSDEQLKSGTASVVCLLNNFYPREAKVQWKVDNALQSGNSQESVTEQDSKDSTYSLSSTLTLSKADYEKHKVYACEVTHQGLSSPVTKSFNRGEC

SEQ ID NO: 24 - protein, 450 aa, synthetic construct
  source 1..450: note = Trastuzumab heavy chain
EVQLVESGGGLVQPGGSLRLSCAASGFNIKDTYIHWVRQAPGKGLEWVARIYPTNGYTRYADSVKGRFTISADTSKNTAYLQMNSLRAEDTAVYYCSRWGGDGFYAMDYWGQGTLVTVSSASTKGPSVFPLAPSSKSTSGGTAALGCLVKDYFPEPVTVSWNSGALTSGVHTFPAVLQSSGLYSLSSVVTVPSSSLGTQTYICNVNHKPSNTKVDKKVEPKSCDKTHTCPPCPAPELLGGPSVFLFPPKPKDTLMISRTPEVTCVVVDVSHEDPEVKFNWYVDGVEVHNAKTKPREEQYNSTYRVVSVLTVLHQDWLNGKEYKCKVSNKALPAPIEKTISKAKGQPREPQVYTLPPSREEMTKNQVSLTCLVKGFYPSDIAVEWESNGQPENNYKTTPPVLDSDGSFFLYSKLTVDKSRWQQGNVFSCSVMHEALHNHYTQKSLSLSPGK

SEQ ID NO: 25 - protein, 214 aa, synthetic construct
  source 1..214: note = Pertuzumab light chain
DIQMTQSPSSLSASVGDRVTITCKASQDVSIGVAWYQQKPGKAPKLLIYSASYRYTGVPSRFSGSGSGTDFTLTISSLQPEDFATYYCQQYYIYPYTFGQGTKVEIKRTVAAPSVFIFPPSDEQLKSGTASVVCLLNNFYPREAKVQWKVDNALQSGNSQESVTEQDSKDSTYSLSSTLTLSKADYEKHKVYACEVTHQGLSSPVTKSFNRGEC

SEQ ID NO: 26 - protein, 449 aa, synthetic construct
  source 1..449: note = Pertuzumab heavy chain
EVQLVESGGGLVQPGGSLRLSCAASGFTFTDYTMDWVRQAPGKGLEWVADVNPNSGGSIYNQRFKGRFTLSVDRSKNTLYLQMNSLRAEDTAVYYCARNLGPSFYFDYWGQGTLVTVSSASTKGPSVFPLAPSSKSTSGGTAALGCLVKDYFPEPVTVSWNSGALTSGVHTFPAVLQSSGLYSLSSVVTVPSSSLGTQTYICNVNHKPSNTKVDKKVEPKSCDKTHTCPPCPAPELLGGPSVFLFPPKPKDTLMISRTPEVTCVVVDVSHEDPEVKFNWYVDGVEVHNAKTKPREEQYNSTYRVVSVLTVLHQDWLNGKEYKCKVSNKALPAPIEKTISKAKGQPREPQVYTLPPSREEMTKNQVSLTCLVKGFYPSDIAVEWESNGQPENNYKTTPPVLDSDGSFFLYSKLTVDKSRWQQGNVFSCSVMHEALHNHYTQKSLSLSPGK

SEQ ID NO: 27 - protein, 8 aa, synthetic construct
  source 1..8: note = CDR1 of HER2-2, HER2-3 and HER2-40
GLTFSTVG

SEQ ID NO: 28 - protein, 8 aa, synthetic construct
  source 1..8: note = CDR2 of HER2-2, HER2-3 and HER2-40
ISWTGNVI

SEQ ID NO: 29 - protein, 12 aa, synthetic construct
  source 1..12: note = CDR3 of HER2-2 and HER2-40
AARRRGTSSYDY

SEQ ID NO: 30 - protein, 25 aa, synthetic construct
  source 1..25: note = FR1 of HER2-2, HER2-3 and HER2-5
QVQLQESGGGLVQAGDSLRLSCAAS

SEQ ID NO: 31 - protein, 17 aa, synthetic construct
  source 1..17: note = FR2 of HER2-2 and HER2-40
MGWFRQLLGKEREPVAA

SEQ ID NO: 32 - protein, 38 aa, synthetic construct
  source 1..38: note = FR3 of HER2-2 and HER2-40
GYGDSVKGRFTISRDSAKNTVYLQMNSLKPEDTAVYYC

SEQ ID NO: 33 - protein, 11 aa, synthetic construct
  source 1..11: note = FR4 of 15 nano antibodies of the present invention
WGQGTQVTVSS

SEQ ID NO: 34 - protein, 8 aa, synthetic construct
  source 1..8: note = CDR1 of HER2-8
GRTFSGAG

SEQ ID NO: 35 - protein, 8 aa, synthetic construct
  source 1..8: note = CDR2 of HER2-8
IAWSGGST

SEQ ID NO: 36 - protein, 20 aa, synthetic construct
  source 1..20: note = CDR3 of HER2-8
AATRRFYSGLTYTQRDVYDN

SEQ ID NO: 37 - protein, 25 aa, synthetic construct
  source 1..25: note = FR1 of HER2-8, HER2-11, HER2-37 and HER2-41
QVQLQESGGGLVQAGGSLRLSCAAS

SEQ ID NO: 38 - protein, 17 aa, synthetic construct
  source 1..17: note = FR2 of HER2-8
VGWFRQDPEKEREFVAA

SEQ ID NO: 39 - protein, 38 aa, synthetic construct
  source 1..38: note = FR3 of HER2-8
RYADSVKGRFTISRDNTENTVFLQMNNLRPEDTAVYYC

SEQ ID NO: 40 - protein, 8 aa, synthetic construct
  source 1..8: note = CDR1 of HER2-10
RNIFGRNV

SEQ ID NO: 41 - protein, 7 aa, synthetic construct
  source 1..7: note = CDR2 of HER2-10
ITGGSAV

SEQ ID NO: 42 - protein, 7 aa, synthetic construct
  source 1..7: note = CDR3 of HER2-10
RAVNDDL

SEQ ID NO: 43 - protein, 25 aa, synthetic construct
  source 1..25: note = FR1 of HER2-10
QVQLQESGGGLVQPGGSLRLSCTAA

SEQ ID NO: 44 - protein, 17 aa, synthetic construct
  source 1..17: note = FR2 of HER2-10
MGWFRQAPGKQREFVAH

SEQ ID NO: 45 - protein, 38 aa, synthetic construct
  source 1..38: note = FR3 of HER2-10
IYATSVKGRFTISRDNAKNTVYLQMNNLTLDDTAVYFC

SEQ ID NO: 46 - protein, 8 aa, synthetic construct
  source 1..8: note = CDR1 of HER2-11
GHTVSRNM

SEQ ID NO: 47 - protein, 8 aa, synthetic construct
  source 1..8: note = CDR2 of HER2-11
IAWNGEDT

SEQ ID NO: 48 - protein, 21 aa, synthetic construct
  source 1..21: note = CDR3 of HER2-11
AASLFRLWNSATAGNNRVYHY

SEQ ID NO: 49 - protein, 17 aa, synthetic construct
  source 1..17: note = FR2 of HER2-11
MGWFRQAPGKEREFVSA

SEQ ID NO: 50 - protein, 38 aa, synthetic construct
  source 1..38: note = FR3 of HER2-11
YYAESVEGRFTISKDNVKNTIYLQMNSLKPEDTAVYYC

SEQ ID NO: 51 - protein, 25 aa, synthetic construct
  source 1..25: note = FR1 of HER2-40
RVQLQESGGGLVQAGGSMRLSCAAS

SEQ ID NO: 52 - protein, 8 aa, synthetic construct
  source 1..8: note = CDR1 of HER2-37
GRTFSSYD

SEQ ID NO: 53 - protein, 8 aa, synthetic construct
  source 1..8: note = CDR2 of HER2-37
IRWRGSIA

SEQ ID NO: 54 - protein, 21 aa, synthetic construct
  source 1..21: note = CDR3 of HER2-37
AATVRTYYGENYDRDASAYGY

SEQ ID NO: 55 - protein, 17 aa, synthetic construct
  source 1..17: note = FR2 of HER2-37
VAWFRQAPEKEREFVAG

SEQ ID NO: 56 - protein, 38 aa, synthetic construct
  source 1..38: note = FR3 of HER2-37
YYVDSVKGRFTISRDNAKNTVYLQMNGLKPEDTAVYYC

SEQ ID NO: 57 - protein, 8 aa, synthetic construct
  source 1..8: note = CDR1 of HER2-38 and HER2-5
ERTFARYV

SEQ ID NO: 58 - protein, 7 aa, synthetic construct
  source 1..7: note = CDR2 of HER2-38 and HER2-5
IYSSGST

SEQ ID NO: 59 - protein, 14 aa, synthetic construct
  source 1..14: note = CDR3 of HER2-38
AARPRDTVWTSSAS

SEQ ID NO: 60 - protein, 23 aa, synthetic construct
  source 1..23: note = FR1 of HER2-38
QLQESGGGLVQAGDSLRLSCAAS

SEQ ID NO: 61 - protein, 17 aa, synthetic construct
  source 1..17: note = FR2 of HER2-38 and HER2-5
MGWFRQAPGKDREFVAH

SEQ ID NO: 62 - protein, 38 aa, synthetic construct
  source 1..38: note = FR3 of HER2-38
AYEGSVKGRFTISRDNAKNTVYLQMNNLKPEDTAVYYC

SEQ ID NO: 63 - protein, 8 aa, synthetic construct
  source 1..8: note = CDR1 of HER2-16
GSIFAFNA

SEQ ID NO: 64 - protein, 7 aa, synthetic construct
  source 1..7: note = CDR2 of HER2-16
ITKEGNT

SEQ ID NO: 65 - protein, 15 aa, synthetic construct
  source 1..15: note = CDR3 of HER2-16
NARDTRKWVSGGYDY

SEQ ID NO: 66 - protein, 25 aa, synthetic construct
  source 1..25: note = FR1 of HER2-16
QVQLQESGGGLVQPGGSLRLSCAPS

SEQ ID NO: 67 - protein, 17 aa, synthetic construct
  source 1..17: note = FR2 of HER2-16
MGWYRQAPGKQRELVAT

SEQ ID NO: 68 - protein, 38 aa, synthetic construct
  source 1..38: note = FR3 of HER2-16
NYVDSVKGRFTISRDNYKNTVDLHMTSLKPDDTAVYYC

SEQ ID NO: 69 - protein, 8 aa, synthetic construct
  source 1..8: note = CDR1 of HER2-41
GRIESSYV

SEQ ID NO: 70 - protein, 8 aa, synthetic construct
  source 1..8: note = CDR2 of HER2-41
IPWSGGAT

SEQ ID NO: 71 - protein, 14 aa, synthetic construct
  source 1..14: note = CDR3 of HER2-41
AARTRDSVWTSSTS

SEQ ID NO: 72 - protein, 17 aa, synthetic construct
  source 1..17: note = FR2 of HER2-41
VGWFRQPPGKEREFVTS

SEQ ID NO: 73 - protein, 38 aa, synthetic construct
  source 1..38: note = FR3 of HER2-41
AYAGSVKGRFTISRDNAKNTLYLQMNNLKPEDTAVYYC

SEQ ID NO: 74 - protein, 8 aa, synthetic construct
  source 1..8: note = CDR1 of HER2-1
GRTFSTYD

SEQ ID NO: 75 - protein, 8 aa, synthetic construct
  source 1..8: note = CDR2 of HER2-1
ITRYGTGP

SEQ ID NO: 76 - protein, 20 aa, synthetic construct
  source 1..20: note = CDR3 of HER2-1
AVQSGIGRVYDYRASVSYTY

SEQ ID NO: 77 - protein, 25 aa, synthetic construct
  source 1..25: note = FR1 of HER2-1
QVQLQESGGGLVQAEGSLRLSCAAS

SEQ ID NO: 78 - protein, 17 aa, synthetic construct
  source 1..17: note = FR2 of HER2-1
IGWFRQAPGKEREFVAR

SEQ ID NO: 79 - protein, 38 aa, synthetic construct
  source 1..38: note = FR3 of HER2-1
LYAGSVKGRFTISRDNAKNTVYLQMNGLKPEDTAVYYC

SEQ ID NO: 80 - protein, 12 aa, synthetic construct
  source 1..12: note = CDR3 of HER2-3
AARRRGMSSYDY

SEQ ID NO: 81 - protein, 17 aa, synthetic construct
  source 1..17: note = FR2 of HER2-3
MGWFRQVLGMEREPVAG

SEQ ID NO: 82 - protein, 38 aa, synthetic construct
  source 1..38: note = FR3 of HER2-3
GYAESVTGRFTISRDSAKNTVYLQMNSLKPEDTAVYYC

SEQ ID NO: 83 - protein, 8 aa, synthetic construct
  source 1..8: note = CDR1 of HER2-4
GRTFIPYD

SEQ ID NO: 84 - protein, 8 aa, synthetic construct
  source 1..8: note = CDR2 of HER2-4
INRLGIGA

SEQ ID NO: 85 - protein, 20 aa, synthetic construct
  source 1..20: note = CDR3 of HER2-4
AAQSGIGAIYDYRASVSYTY

SEQ ID NO: 86 - protein, 25 aa, synthetic construct
  source 1..25: note = FR1 of HER2-4
QVQLQESGGGLVPAEGSLRLSCAAS

SEQ ID NO: 87 - protein, 17 aa, synthetic construct
  source 1..17: note = FR2 of HER2-4
IGWFRQAPGKEREFVAH

SEQ ID NO: 88 - protein, 38 aa, synthetic construct
  source 1..38: note = FR3 of HER2-4
LYAGSVEGRVTISRDNVKNTVYLQMNGLKPEDTAVYYC

SEQ ID NO: 89 - protein, 15 aa, synthetic construct
  source 1..15: note = CDR3 of HER2-5
AARDRDSTWNQGTSH

SEQ ID NO: 90 - protein, 38 aa, synthetic construct
  source 1..38: note = FR3 of HER2-5
AYEGSVKGRFTISRDNAKNTVYLQMNSLKPEDTAVYYC

SEQ ID NO: 91 - protein, 8 aa, synthetic construct
  source 1..8: note = CDR1 of HER2-32
GGTISTDV

SEQ ID NO: 92 - protein, 8 aa, synthetic construct
  source 1..8: note = CDR2 of HER2-32
IQWSRDYT

SEQ ID NO: 93 - protein, 16 aa, synthetic construct
  source 1..16: note = CDR3 of HER2-32
ARHWSGDIYASNSYNS

SEQ ID NO: 94 - protein, 25 aa, synthetic construct
  source 1..25: note = FR1 of HER2-32
QVQLQESGGGLVQAGGSLRLTCAAS

SEQ ID NO: 95 - protein, 17 aa, synthetic construct
  source 1..17: note = FR2 of HER2-32
MGWFRQDPGKEREFVAA

SEQ ID NO: 96 - protein, 38 aa, synthetic construct
  source 1..38: note = FR3 of HER2-32
YYSDSVKGRFTGSRDNAKNTVYLQMNSLKPEDAAVYYC

SEQ ID NO: 97 - protein, 8 aa, synthetic construct
  source 1..8: note = CDR1 of HER2-34
RSIFNALM

SEQ ID NO: 98 - protein, 6 aa, synthetic construct
  source 1..6: note = CDR2 of HER2-34
TRGGST

SEQ ID NO: 99 - protein, 7 aa, synthetic construct
  source 1..7: note = CDR3 of HER2-34
RDWGHDS

SEQ ID NO: 100 - protein, 25 aa, synthetic construct
  source 1..25: note = FR1 of HER2-34
QVQLQESGGGLVQPGGSLNLSCAAS

SEQ ID NO: 101 - protein, 17 aa, synthetic construct
  source 1..17: note = FR2 of HER2-34
GWYRQAPGNQREFVAHI

SEQ ID NO: 102 - protein, 38 aa, synthetic construct
  source 1..38: note = FR3 of HER2-34
MYADSVKGRFTISRDNAKNTVYLQMNGLKPDDSAVYYC